European Patent Specification EP 4 322 973 B1, published June 4, 2025. Title: Hyperimmunized Egg Product for Treating or Preventing Alcoholic Liver Disease and Graft-versus-Host Disease. Applicant: Iyer, Subramanian V Patel, Sunny. The sequence listing filed with the application follows.

SEQUENCE LISTING (2 sequences)

SEQ ID NO: 1 - protein, 38 aa, Enterococcus faecalis
TTPVCAVAATAAASSAACGWVGGGIFTGVTVVVSLKHC

SEQ ID NO: 2 - protein, 21 aa, Enterococcus faecalis
TTPACFTIGLGVGALFSAKFC